European Patent Specification EP 3 722 433 B1, published July 26, 2023. Title: PROMOTER AND REGULATORY ELEMENTS FOR IMPROVED EXPRESSION OF HETEROLOGOUS GENES IN HOST CELLS. Applicant: Amgen Inc. Application not yet assigned. The sequence listing filed with the application follows.

SEQUENCE LISTING (54 sequences)

SEQ ID NO: 1-8 - skipped (8 entries)

SEQ ID NO: 9 - DNA, 29 bp, ARTIFICIAL SEQUENCE
  Forward Primer
ctacccagagacctatttctgtcatagcc

SEQ ID NO: 10 - DNA, 19 bp, ARTIFICIAL SEQUENCE
  Reverse Primer
ccaggcgtccaatacggcc

SEQ ID NO: 11 - DNA, 4210 bp, Cricetulus griseus
  misc_feature: Chinese hamster GAPDH gene, -2049 through +2161 relative to transcription start site
ctacccagagacctatttctgtcatagccttttgggacacataaagcttccttcctgcatagaacaccccacaacagtgtatcaggagtgtacaagttgacaaacaatgctctagacctacggttttcttcctctgtgtgcctcatcccagaagagatcatgactcccaggagtcagcctttactatggggtctgcaggggcgtccagcccctcagcggcaagccatgcccaccctccccaagtccttaatctgctgagtcacttggaacaggagacactgattctgctgtcatgacaacagcacattgccatagaaatgctccctacctcttacgtgtgtggtgggggaacagtaatgacaaaccataggcaggaggcaaaagggaagacggcacctcagaaacatgtgttaggttagggcagaactatggaggggctcctgagactctttgatgggaaagggttaatgctgctcctgaaacctctgttggaaggcagaaaagggacagggctgagtccccgcactgggaccatttccatcctctgcatcctgcccccggctcatggaaagcctgggcatgggccacacagctgtcagtcttggctctggggccccaaggaggtagggcaatcccagaatggcaaggagccaggactggatttggggtgcagcccagcctgctccctgccttttaagcaaaggttatcaccaggccagctaaacttagcaattaggctcttcagctaaaagagcagggggctggtctcaagttgcactgacctagcaaagaggccccaggatccccctgcccagcacctgtggctgagctcccaagcccttcccgagagctcaggatccaccctttccaccctccctactcttcagaggaggaaccccctttctccttcccacttgttggagggggctggggccaggctgttctggcttggggtataataccccctaccccttctactttcccctcctctcagacctcaccctgcctccacgagggcagccaagaaaggagagtccctggctgcagggccagtaggcacgtcccaggacggggagggacttccgccctcacgtccagctctccgccctggggctgcagtgggtgaaaggggcagtgtctcctagcctgggcggtgcaaccctcaggttccgaggaggaacgctctgggaggcttctttgcctcctccaacccaacccacaaccaggacattgtcctcaccccggggccccaacctagaccttaactgaggaacacagaggccagtttgtaagtctcaattatgcagggcatcccgacctgtggcgtagggagcgcccctccaggccgcttccctagcctcctcctggccctcacagcccaggcctctggcccaagaaatggaagtgggggtgggggatggaactgcgaatgcgaagggcccccgcaggaggcaaagtgacccctcccgggccttttctgctccgagacttgtttttgcctgtgtcactaccgaagaaccacgagaagatcctcaacttttccacagcctttgcataaaggggagagggtcggcggtgcagctgtggcacacacgcacttctgctcaacccgcccccccccgcccccgttcctgttccttcccaggttctccccattttatcggggcggcaacttttaggtccctgggtcctggaagtccttagtacacactcttcgtccttaagtccatagtctgtattccctcggtcctatcctgtcccccatcaccgggtcacctccccagcgaagcaatctcagttcccctccccctctcagccccgagcccacacgtttggtgcgtgcacatttcaaaaacgaggcgggtccaaagagagggggtggggaggtgccgagtggcccagctactcgcggctttacgggtgcacgtagctcaggcctcagcgcccttgagctgtgactggatggatgagcggggcgggaggcggggcgagcgtcctcggcgctccccaccaccccagttcctataaatacggactgcagccctccccggtgctctctgctcctccctgttctagagacagccgcatctttccgtgcagtgccaggtgaaaaccgcagagtgggccgcaggtggccggggacggtcggaaacggggaaggggggcgctcagcccgggactgcgggcgctggggcgagctccactgcccgagcccgggctccgcattgcagaggctggagggggacgtgatggggcgcgcggcgggaatggaggcgggggggggggtcgccctgtgaccgtggtccacgctgacctctctttcttctctctccctccgcagcctcgctccggagacgcaatggtgaaggtcggcgtgaacgggtgagttcgtggctgggctagggtggggctccgggtcccgctccgtcgcgtatgcaggtctaccccaccccggggctctgcgggagcgtggggtggccggtgggtggccgcagcacccaaggagacctcaaggtcagcgagccggctccgcccttgcggggatgagcagcgcggagtcctcacgaggaggaccatcccccgcgcgcacgcatgcttaggctccatcccgatccccagccgggggcttctttctttactttcgcgccctgaggaaccacgtgccagacgggagcccctcccccattgccctctacccccccccccgcgcgcgcctccaggtcggtggcaccgggccgtgcggtgcccgctttagcgcatccatcatctcccaagggcttcctttagggtggctggccgccgccatgttgcaaacgggaaggaaatgaatgaaccaccgttaggaaacctcccttcggccttcctccttcctagcccgtgactaacctccccactccctccccgggtggagtcgcctctgtactgtaagccaggtgatgcaaggcttccgtgctctcgagagagctctacctcgccagctgtctcatattattagcctcaaagcagccctcaagcctcatttaccttgagcatatgatatattttgtagattctctgagaatcgaagcggacttggagaggtctgcttgtccttctcccagcccaaaggtggtagctatggcgtagcgccggaggggggagtggggggggagctgagtcatggtggttctgaaaagaaaatttccaccacaaaatggctccggtgctagcatccccttccccccataacctctgcttcccatcacaccctgacccaaaccctgtaggccagactgtaaaggtcactaagaggattgagtgtctgagcctcggaaccctgcccttctccccatcccatcctctggaaaccagatctcccccgctccaccctaatctgaggttatatttagccggctgacctttcagtatttggggtctgggcccctacacacatctgttgctcctgctcctgatttttagctagcaaattcaagtgctttgcaaattagagcccagggattaggggttggaaagctcagtggttttctcagtctttccctttagggggagggacttggaggaagcaggtgggccgacccctgtcctactcattctgacctttaaccttgccctttgagcttgatgatgctgagtgcacgagttcttcctgtccagggggtgtagcctgaagccaggccaggctagaacaaacttcccagggggtgggggtagtgaatgccttgtgcccacacaggggcacactgccacctcttggagacttgaaatgactggtgggggggttggacaaggctttgagcccaatcacctcttggacaggaaagtaacccccactttatggccctgctgtaaaagcccagtcaaacctcatttgtccaaggaagatagacctcttggggcttcctaaggataggggtgttctatatttgggccctgcttctaagcattcagccagctttattaaaggaaattcataacaaaacttgaatttcctgcttcttaaatactaatagtgtgctggatctccattaaaaatgctgtcttgcacagtaggctatggtttctgtgggctctctacagctatgggacaactggattctgttttctgaagggcatgtgtcagctcagtactgactatagacctatgagttctctgaccccctaactcacctttttttttcttgcctcagatttggccgtattggacgcctgg

SEQ ID NO: 12 - DNA, 24 bp, ARTIFICIAL SEQUENCE
  Forward Primer 4
gatagttggcatttgctgttctag

SEQ ID NO: 13 - DNA, 38 bp, ARTIFICIAL SEQUENCE
  Reverse Primer 4
tgtaacggatccagacttcaacacatctatttttctac

SEQ ID NO: 14 - DNA, 38 bp, ARTIFICIAL SEQUENCE
  Forward Primer 5
tgaagtctggatccgttacataacttacggtaaatggc

SEQ ID NO: 15 - DNA, 25 bp, ARTIFICIAL SEQUENCE
  Reverse Primer 5
ccatggtaatagcgatgactaatac

SEQ ID NO: 16 - DNA, 46 bp, ARTIFICIAL SEQUENCE
  Forward Primer 6
gtcatcgctattaccatggcctcgagaccacgagaagatcctcaac

SEQ ID NO: 17 - DNA, 45 bp, ARTIFICIAL SEQUENCE
  Reverse Primer 6
cattccatggtggcctagtcgacgctagcctccggagcgaggctg

SEQ ID NO: 18 - DNA, 33 bp, ARTIFICIAL SEQUENCE
  Reverse Primer 7
cgagctctgcttatataggaactggggtggtgg

SEQ ID NO: 19 - DNA, 32 bp, ARTIFICIAL SEQUENCE
  Forward Primer 7
gttcctatataagcagagctcgtttagtgaac

SEQ ID NO: 20 - DNA, 47 bp, ARTIFICIAL SEQUENCE
  Reverse Primer 8
cattccatggtggcctagtcgacgctagcaggttttccgatccggtc

SEQ ID NO: 21 - DNA, 27 bp, ARTIFICIAL SEQUENCE
  Reverse Primer 9
cggtactcaccccaacagctggccctc

SEQ ID NO: 22 - DNA, 29 bp, ARTIFICIAL SEQUENCE
  Forward Primer 8
ctgttggggtgagtaccgcagagtgggcc

SEQ ID NO: 23 - DNA, 26 bp, ARTIFICIAL SEQUENCE
  Reverse Primer 10
ccgcgagctgcggagggagagagaag

SEQ ID NO: 24 - DNA, 28 bp, ARTIFICIAL SEQUENCE
  Forward Primer 9
cctccgcagctcgcggttgaggacaaac

SEQ ID NO: 25 - DNA, 29 bp, ARTIFICIAL SEQUENCE
  Reverse Primer 11
gaactcacctgaggttttccgatccggtc

SEQ ID NO: 26 - DNA, 28 bp, ARTIFICIAL SEQUENCE
  Forward Primer 10
cggaaaacctcaggtgagttcgtggctg

SEQ ID NO: 27 - DNA, 47 bp, ARTIFICIAL SEQUENCE
  Reverse Primer 12
cattccatggtggcctagtcgacgctagccaaatctgaggcaagaaa

SEQ ID NO: 28 - DNA, 21 bp, ARTIFICIAL SEQUENCE
  Forward Primer 11
gatgtgttgaagtctggatcc

SEQ ID NO: 29 - DNA, 27 bp, ARTIFICIAL SEQUENCE
  Reverse Primer 13
caaccgcgagcccaacagctggccctc

SEQ ID NO: 30 - DNA, 30 bp, ARTIFICIAL SEQUENCE
  Forward Primer 12
gctgttgggctcgcggttgaggacaaactc

SEQ ID NO: 31-32 - skipped (2 entries)

SEQ ID NO: 33 - DNA, 23 bp, ARTIFICIAL SEQUENCE
  Forward Primer
gattagaagccatcttgttacaa

SEQ ID NO: 34 - DNA, 25 bp, ARTIFICIAL SEQUENCE
  Reverse Primer
tatataactctgaaagtgtcaaccc

SEQ ID NO: 35 - DNA, 3045 bp, Cricetulus griseus
  misc_feature: Rps3 genomic fragment
gattagaagccatcttgttacaaatgtcaaaagatcattcctgttttctgtaatacttgtgtttgaccatgtcttgatccatcttctggaatttgacatgttccacaccttataccctgacctccatcctgacaagataagatgttctgccactgtcctacataaccaaaatgcctcttcaaatcgcccaatccttgaaatttctgagctatataaattctactttcttctatgtccaatgctgttttttcaaactccactttagggagacaaccctgtttgacagaaaataaaacttccttaatctaactaaaacaatttgggtaatgggctttacttttatttggtgggatttgcacagggtgaattggagccccctggagatgactgagccacgaacactgtagtacaagttactgaagcaggatttgcttctggacaaggagtgattgctggtgtagacatcggagtccctgtgaagggatgtcctgtggcccagacttacactttctgataatctgtcttcaaagccctgctagtttattacattgacagctcccttctggtagcccaccccactgtgagttcaaaaagttcagaggtcctggtgcaagtgtttgataccagaaatgctacaggtaagtccatctttaggatcagggtttatctttgtaataaacatcataggattgtaatgttttaacaatgacgtgtgtgtgtgtgtgtgtgtgtgtgtgtgtgtgtgtgtgtgtgtgtgtgtttgtgtttgtgtggggagagcatgcatgggaaggtcctaggacctaggttctgtcctttgacctctgggtgctgggatcgaaatcaaacacctttacctactaagtcacctggctggtcccccaaatgaatttcaatgagagttttcattagtgtggtcctgaagctataagcaatagggttccagtctgggtaaactctgttagtgtatgcttatgtctgtggtttgcatctcttgcctcttggttgctctgttcaaagtttttatttatttttgagtcgggggctcatgtagaccaagctggcttcgaactcgctatgtagtcgagaatgaccttgaatttttgattctccagcctccacctctctagtgctgaaatcactggtgtgctcctccacggtggggtacattgattgtttttcagaccagaattagatttgcacttcctgttccgcctacactacgggttgctaggttacacttctttttctcttttcgcctttataaactcaaaacttcatttcccatgagctcttgcaagtgtcgccgttgcgtggcgttgcgtcgtcgttccgcgccctttatacacacttccgcccgcgagctacttcctttcctttcggtggcgcgcggcggcaagatggcggtgcagatttccaagaagaggaaggtaagcatttcggaccggctcggggactcgcggcgcgttttaaagctgccacggtgagacccgcagctccgtgtccgatcccggagagcggctactgccgcctggcgcttccgcggggcgcggatggacgtggattgtgtgctgggccggctccgggctagctcagtgtggctgaggaagggaggaacagacgcctcagttctgggccgaggtgaacactggaagccatcaggcctttactagacgcttttgagcgtctctcggtcgccagaattagtaaccctatggcatagcttgagagcgtgagctaatccggcgtctttggtaagtgaggtttagcagtgccgcctcagttgaaaggctgccgactattggcgtgctccctcgggacctgcagcaaaagcgtcccggacttttgtcatttcatggggaagaagtgtgtgaagatcatcaggtttagaaatagatggcctgtctttgtgatcaagcacatagatcataaagctgttgtccacatgctgtttgggttagatttgtcctctcttgcttcaggtacgagttacatacacacacggtgttcttgctgtgctgtgtgaactgcagatgtgctacttgaatagatttttgttctgtgtgtgtaaatgttttaaaacccttcgatgaagaggtgatgacgagtctgacggaggtgttgtctttgtccaaaaggcgtcactgtgctgcgttctgtggcacagctgaaagcactatggtcaaaggaacttcctaaagatgacctagaggcatttgtctgagaagggttgctgcattcccgaagggtcattggggtcgaactgggtaagcctctaccctttcttaactctgaacttgcttttggtttagtttgtggctgatggcatcttcaaagcagagctgaatgagtttctcactcgggaactggctgaagacggctactcgggagttgaagtccgagttacaccaaccagaacagaaatcattattttagccaccaggtaaaaatatgtttgactggctattacctgtaatcactgtgtgtattgagttgctgtgtaaacttggaacaaccaaccagtgaacctgctccttttttgttgttgttttttgtttgttttttgagacagggtttctctgcattgcttgggagcctggcctggaacttgctctgtggatcagtctggcctaagactcacagagatccgcctgctctgcctcctgagtgctgggattaaaggtgtgcaccaccaccactgcctggccttggagttgcttttttaaaacaccatttgtaaagaatttaccttaatacttttttaaagtgtgtccttgctgtgtgataaatggtatgtgaggtgttgcaaataaattgtaattttcccttctgcagaacacaaaatgttcttggtgagaagggtcgtcgaatcagagagttgactgcggtagttcagaagaggttcggcttccctgagggcagcgtagaggtgagtttccctggtttataccaggggcagtagactggatttagaagttgcttctgtagaacggtaattctggacaatgagtagtacaggtgggttgacactttcagagttatata

SEQ ID NO: 36 - DNA, 22 bp, ARTIFICIAL SEQUENCE
  Forward Primer
caaagaggttgagatcgtaccc

SEQ ID NO: 37 - DNA, 18 bp, ARTIFICIAL SEQUENCE
  Reverse Primer
tgagaccgctgccaaagc

SEQ ID NO: 38 - DNA, 3258 bp, Cricetulus griseus
  misc_feature: Rps2 genomic fragment
caaagaggttgagatcgtacccaccactctgcaaaggccaagttagtgttaaagtctgtcccaaagcacacataccatcaagataactccataatcattctgtagggaggcaggctacataaagaaactcaagggcaaacctgtgggggttgagtcccccaagatttgccaatatttgactgaagaagctggaataccacctagagccttctgaaatgttttcttgccccataaaggaactatcattcattcgcagagtgagacaggatcgattcctagacagctgggcagctgtctggaattgagtacatatctcagagctggtggaaagaagccagggcctcaccatgatctgtgtctggacggcagctccactgaggccaagggcttaggagcctccatttcacagtacatgtggaccgacatcacagtggcattgtctagcttgagccaatcacagctctggtccagagccaattgggaccttgtggctaccttaccctttgccttgccctctgaaggtgagtggtagggtggcctcaactcaggagtagtctatggattctcttgcttgccttggttgtggctgacagctgagcccaagcttctagggactggttcccaaggccagtaggatcccagggattgtagcctcctccattgactgggtggtcagtttagatgttggtcctgctccacaaacatcccttcaccaagaattaagcccaatagcaagagccacattctttgaaagagaccagaggcttttcagtttaacttaaaggcctttggggactgggcagtggtagtgcaagcaaagcctttaatcctagcacaaacgagacagaggtagttgtatctgtgattttgaggccagcctgatctacagagtgagttctaggacagctagagctgtttcacagagaaaccctgtctggaagaaataaaacaaaaggccttggagagataagctttagaatacatgctttagtgtagttctttttgtgtataacatggtttccatattggcatagagatcacactgggcagataaccatattaactgagcagaaagaatataaagtaggcctaagggaacattagtggagctactgacaatcctctccttcagctgcaatctattttgggagatgcctgagtatacacaaagtaaaagggccactccatgattaagtgtccaggtcataatcctcgattgggtaggactgtttgctgtttcagggccacacacgctcaataacgcttcatgaagttgaacttgagtggaatcatactttggccatcactagtgcactatttggggtgaacagatgtcttccctagaaggggaaatgccaacacactacttctaggtggtcatgtaaaaatttttgaaatagaccgggcattggtggcacacacctttattcctaccactcaggaggcagaggcaggtggatctctgtgaatttgcaatcagcctggtctacaagccctagttgcaaggcagcctccaaagtcacagagaaaccctgtcttgaacgcaccccccccccccccccccgcccaattttttttttttaaaataacctggctggagagatggctcagaagttaagagcactgactgcccttccggaggtcctgagttcaattccaggcaaccttatggtggctcaaaaccatctgtaatgagatttggcgccctcttctggcatgcaacatacatgttggtagcacactgtatatataataaataaatcttgtctctgactctcagtgcaagcaaccacacccaagctccagtcatttaaagaagccaaacactgaaaccaatgggagctcctgtagcatccttgttctgctgcttgatgatcactctggatgaggaatacctgtgtggtgcacagtacatctggagcatgagtacaagacaaggcctaacccagatgaaacttgtcacatacacatttctacctgtgtagtgacatttggaaggccgaagcaggattgttaaattccatgtcctcactgaatacacagcaggacccactctcaaaacaaaacaaaacttagggttcaactatacgaaactccagttccaggggctcagatatctttttacggccacaggcatcagacaacgtggtgcatatacattcatgcaggcaaaataaaagcgcacttaaagaaaagctggaatctagcagggtggaatctaacttacaggggtctggctgcgtcggccatccagatgctacctgttgggactaacacacccgccacgaatacgtttttcacctagattgacagaaaccctccaagaaaaccagaagaaaaacacaaacaaaacaccaccaccaccacatacacggtaggttatgttaaaccactttatttgagaagaggacatcggaaccctgccattttcgtgggcgaagctgcagccgcctccagatccagtggaacctgtggataaaggacatggttaggatcgatgccacacacaagccaggccgcgggagccgcgaggcggtcgggaatgtaggggcctgggtttcaccctcccacactggggcagcgggcggtgagctgaggcccctgtggctctgggcgccgaatctcacctccggccacagccaaggccgaaaatgattttcaacgaacgcccatttaccgagcccacggcgaacgcgaggctgacgaggtacaacctacctgaggcagagagaaagagcaggaagtgacgagcactaggaggcctgagaggcgccacccggacttttatacaccctcacagtcggcgtacgtcgcggcttcggcgaggcgatatgcgcaggcgcagatggaacgtgcggggcgggggggggggaggtgacaacacgcagccaattacagcctgcgtgtgagctgagcaggcctggagatatcgcggcgctaggggcactataaagtctgccttccccacagccgcgctcttcttctacttcgggaaaacacgtgagtcgttgttcctcagtcccggtgtcggggcctgggcagtgggaatccgtggacatccggacggagacgcccttgggcgggaggtcccctatcggaatcccaagcgaccgcaaagccaattgtcgttctgagttgcttttttgcttctctagcaaatggcggatgacgccggtgcagctggagggcccggaggacccgggggcccaggattaggaggtcgcggaggcttccgcggaggctttggcagcggtctca

SEQ ID NO: 39 - DNA, 37 bp, ARTIFICIAL SEQUENCE
  Forward Primer
ggaattagacggatcccaaagaggttgagatcgtacc

SEQ ID NO: 40 - DNA, 39 bp, ARTIFICIAL SEQUENCE
  Reverse Primer
cgtaagttatgtaacggatcctgagaccgctgccaaagc

SEQ ID NO: 41 - DNA, 34 bp, ARTIFICIAL SEQUENCE
  Forward Primer
ggaattagacggatcctgagaccgctgccaaagc

SEQ ID NO: 42 - DNA, 42 bp, ARTIFICIAL SEQUENCE
  Reverse Primer
cgtaagttatgtaacggatcccaaagaggttgagatcgtacc

SEQ ID NO: 43 - DNA, 23 bp, ARTIFICIAL SEQUENCE
  Forward Primer
caacttacttctgacaacgatcg

SEQ ID NO: 44 - DNA, 29 bp, ARTIFICIAL SEQUENCE
  Reverse Primer
ggatccgtctaattccggtctccctatag

SEQ ID NO: 45 - DNA, 40 bp, ARTIFICIAL SEQUENCE
  Forward Primer
ggaattagacggatccgattagaagccatcttgttacaaa

SEQ ID NO: 46 - DNA, 46 bp, ARTIFICIAL SEQUENCE
  Reverse Primer
cgtaagttatgtaacggatcctatataactctgaaagtgtcaaccc

SEQ ID NO: 47 - DNA, 42 bp, ARTIFICIAL SEQUENCE
  Forward Primer
ggaattagacggatcctatataactctgaaagtgtcaaccca

SEQ ID NO: 48 - DNA, 45 bp, ARTIFICIAL SEQUENCE
  Reverse Primer
cgtaagttatgtaacggatccgattagaagccatcttgttacaaa

SEQ ID NO: 49 - DNA, 837 bp, Cricetulus griseus
  misc_feature: GAPDH gene fragment (-532 through +305)
accacgagaagatcctcaacttttccacagcctttgcataaaggggagagggtcggcggtgcagctgtggcacacacgcacttctgctcaacccgcccccccccgcccccgttcctgttccttcccaggttctccccattttatcggggcggcaacttttaggtccctgggtcctggaagtccttagtacacactcttcgtccttaagtccatagtctgtattccctcggtcctatcctgtcccccatcaccgggtcacctccccagcgaagcaatctcagttcccctccccctctcagccccgagcccacacgtttggtgcgtgcacatttcaaaaacgaggcgggtccaaagagagggggtggggaggtgccgagtggcccagctactcgcggctttacgggtgcacgtagctcaggcctcagcgcccttgagctgtgactggatggatgagcggggcgggaggcggggcgagcgtcctcggcgctccccaccaccccagttcctataaatacggactgcagccctccccggtgctctctgctcctccctgttctagagacagccgcatctttccgtgcagtgccaggtgaaaaccgcagagtgggccgcaggtggccggggacggtcggaaacggggaaggggggcgctcagcccgggactgcgggcgctggggcgagctccactgcccgagcccgggctccgcattgcagaggctggagggggacgtgatggggcgcgcggcgggaatggaggcgggggggggggtcgccctgtgaccgtggtccacgctgacctctctttcttctctctccctccgcagcctcgctccggag

SEQ ID NO: 50 - DNA, 510 bp, Cricetulus griseus
  misc_feature: GAPDH promoter (-532 through -23)
accacgagaagatcctcaacttttccacagcctttgcataaaggggagagggtcggcggtgcagctgtggcacacacgcacttctgctcaacccgcccccccccgcccccgttcctgttccttcccaggttctccccattttatcggggcggcaacttttaggtccctgggtcctggaagtccttagtacacactcttcgtccttaagtccatagtctgtattccctcggtcctatcctgtcccccatcaccgggtcacctccccagcgaagcaatctcagttcccctccccctctcagccccgagcccacacgtttggtgcgtgcacatttcaaaaacgaggcgggtccaaagagagggggtggggaggtgccgagtggcccagctactcgcggctttacgggtgcacgtagctcaggcctcagcgcccttgagctgtgactggatggatgagcggggcgggaggcggggcgagcgtcctcggcgctccccaccaccccagttcctata

SEQ ID NO: 51 - DNA, 231 bp, Cricetulus griseus
  misc_feature: GAPDH intron 1 (+64 through +293)
accgcagagtgggccgcaggtggccggggacggtcggaaacggggaaggggggcgctcagcccgggactgcgggcgctggggcgagctccactgcccgagcccgggctccgcattgcagaggctggagggggacgtgatggggcgcgcggcgggaatggaggcgggggggggggtcgccctgtgaccgtggtccacgctgacctctctttcttctctctccctccgcagcc

SEQ ID NO: 52 - DNA, 1812 bp, Cricetulus griseus
  misc_feature: GAPDH intron 2 (+334 through +2145)
gtgagttcgtggctgggctagggtggggctccgggtcccgctccgtcgcgtatgcaggtctaccccaccccggggctctgcgggagcgtggggtggccggtgggtggccgcagcacccaaggagacctcaaggtcagcgagccggctccgcccttgcggggatgagcagcgcggagtcctcacgaggaggaccatcccccgcgcgcacgcatgcttaggctccatcccgatccccagccgggggcttctttctttactttcgcgccctgaggaaccacgtgccagacgggagcccctcccccattgccctctacccccccccccgcgcgcgcctccaggtcggtggcaccgggccgtgcggtgcccgctttagcgcatccatcatctcccaagggcttcctttagggtggctggccgccgccatgttgcaaacgggaaggaaatgaatgaaccaccgttaggaaacctcccttcggccttcctccttcctagcccgtgactaacctccccactccctccccgggtggagtcgcctctgtactgtaagccaggtgatgcaaggcttccgtgctctcgagagagctctacctcgccagctgtctcatattattagcctcaaagcagccctcaagcctcatttaccttgagcatatgatatattttgtagattctctgagaatcgaagcggacttggagaggtctgcttgtccttctcccagcccaaaggtggtagctatggcgtagcgccggaggggggagtggggggggagctgagtcatggtggttctgaaaagaaaatttccaccacaaaatggctccggtgctagcatccccttccccccataacctctgcttcccatcacaccctgacccaaaccctgtaggccagactgtaaaggtcactaagaggattgagtgtctgagcctcggaaccctgcccttctccccatcccatcctctggaaaccagatctcccccgctccaccctaatctgaggttatatttagccggctgacctttcagtatttggggtctgggcccctacacacatctgttgctcctgctcctgatttttagctagcaaattcaagtgctttgcaaattagagcccagggattaggggttggaaagctcagtggttttctcagtctttccctttagggggagggacttggaggaagcaggtgggccgacccctgtcctactcattctgacctttaaccttgccctttgagcttgatgatgctgagtgcacgagttcttcctgtccagggggtgtagcctgaagccaggccaggctagaacaaacttcccagggggtgggggtagtgaatgccttgtgcccacacaggggcacactgccacctcttggagacttgaaatgactggtgggggggttggacaaggctttgagcccaatcacctcttggacaggaaagtaacccccactttatggccctgctgtaaaagcccagtcaaacctcatttgtccaaggaagatagacctcttggggcttcctaaggataggggtgttctatatttgggccctgcttctaagcattcagccagctttattaaaggaaattcataacaaaacttgaatttcctgcttcttaaatactaatagtgtgctggatctccattaaaaatgctgtcttgcacagtaggctatggtttctgtgggctctctacagctatgggacaactggattctgttttctgaagggcatgtgtcagctcagtactgactatagacctatgagttctctgaccccctaactcacctttttttttcttgcctcagatttggc

SEQ ID NO: 53 - protein, 66 aa, ARTIFICIAL SEQUENCE
  VK-1 signal peptide coding sequence
ATGGACATGAGGGTGCCCGCTCAGCTCCTGGGGCTCCTGCTGCTGTGGCTGAGAGGTGCGCGCTGT

SEQ ID NO: 54 - protein, 22 aa, ARTIFICIAL SEQUENCE
  VK-1 signal peptide sequence
MDMRVPAQLLGLLLLWLRGARC